European Patent Application EP 4 756 014 A1, published June 10, 2026. Title: Cell therapeutic agent based on recombinant immune cells for treating cancer via polyclonal expansion of tumor-infiltrating T cell in tumor. Applicant: Korea Advanced Institute of Science and Technology. The sequence listing filed with the application follows.

SEQUENCE LISTING (20 sequences)

SEQ ID NO: 1 - protein, 141 aa, synthetic construct
MNSGLQLVFFVLTLKGIQGEVQLVESGGGLVQPGKSLKLSCEASGFTFSGYGMHWVRQAPGRGLESVAYITSSSINIKYADAVKGRFTVSRDNAKNLLFLQMNILKSEDTAMYYCARFDWDKNYWGQGTMVTVSSAKTTAP

SEQ ID NO: 2 - DNA, 423 bp, synthetic construct
  source 1..423: mol_type = other DNA
atgaactcaggactccaattggttttctttgtcctcactctaaaaggtatacagggtgaggtgcagctggtggagtctgggggaggcttggtgcagcctggaaagtccctgaaactctcctgtgaggcctctggattcaccttcagcggctatggcatgcactgggtccgccaggctccagggagggggctggagtcggtcgcatacattactagtagtagtattaatatcaaatatgctgacgctgtgaaaggccggttcaccgtctccagagacaatgccaagaacttactgtttctacaaatgaacattctcaagtctgaggacacagccatgtactactgtgcaagattcgactgggacaaaaattactggggccaaggaaccatggtcaccgtctcctcagccaaaacaacagcccca

SEQ ID NO: 3 - protein, 108 aa, synthetic construct
DIQMTQSPSSLPASLGDRVTINCQASQDISNYLNWYQQKPGKAPKLLIYYTNKLADGVPSRFSGSGSGRDSSFTISSLESEDIGSYYCQQYYNYPWTFGPGTKLEIKR

SEQ ID NO: 4 - DNA, 324 bp, synthetic construct
  source 1..324: mol_type = other DNA
gacatccagatgacccagtctccatcatcactgcctgcctccctgggagacagagtcactatcaattgtcaggccagtcaggacattagcaattatttaaactggtaccagcagaaaccagggaaagctcctaagctcctgatctattatacaaataaattggcagatggagtcccatcaaggttcagtggcagtggttctgggagagattcttctttcactatcagcagcctggaatccgaagatattggatcttattactgtcaacagtattataactatccgtggacgttcggacctggcaccaagctggaaatcaaacgg

SEQ ID NO: 5 - protein, 119 aa, synthetic construct [sequence omitted]

SEQ ID NO: 6 - DNA, 357 bp, synthetic construct
  source 1..357: mol_type = other DNA
caggtccagctgcagcagtctggggctgaactggcaagacctggggcctcagtgaagatgtcctgcaaggcttctggctacacctttactaggtacacgatgcactgggtaaaacagaggcctggacagggtctggaatggattggatacattaatcctagccgtggttatactaattacaatcagaagttcaaggacaaggccacattgactacagacaaatcctccagcacagcctacatgcaactgagcagcctgacatctgaggactctgcagtctattactgtgcaagatattatgatgatcattactgccttgactactggggccaaggcaccactctcacagtctcctca

SEQ ID NO: 7 - protein, 107 aa, synthetic construct
QIVLTQSPAIMSASPGEKVTMTCSASSSVSYMNWYQQKSGTSPKRWIYDTSKLASGVPAHFRGSGSGTSYSLTISGMEAEDAATYYCQQWSSNPFTFGSGTKLEINR

SEQ ID NO: 8 - DNA, 321 bp, synthetic construct
  source 1..321: mol_type = other DNA
caaattgttctcacccagtctccagcaatcatgtctgcatctccaggggagaaggtcaccatgacctgcagtgccagctcaagtgtaagttacatgaactggtaccagcagaagtcaggcacctcccccaaaagatggatttatgacacatccaaactggcttctggagtccctgctcacttcaggggcagtgggtctgggacctcttactctctcacaatcagcggcatggaggctgaagatgctgccacttattactgccagcagtggagtagtaacccattcacgttcggctcggggacaaagttggaaataaaccgg

SEQ ID NO: 9 - protein, 333 aa, synthetic construct
METDTLLLWVLLLWVPGSTGDYPYDVPDYAGGGGSGGGGSDIQMTQSPSSLPASLGDRVTINCQASQDISNYLNWYQQKPGKAPKLLIYYTNKLADGVPSRFSGSGSGRDSSFTISSLESEDIGSYYCQQYYNYPWTFGPGTKLEIKRGGGGSGGGGSGGGGSEVQLVESGGGLVQPGKSLKLSCEASGFTFSGYGMHWVRQAPGRGLESVAYITSSSINIKYADAVKGRFTVSRDNAKNLLFLQMNILKSEDTAMYYCARFDWDKNYWGQGTMVTVSSGGGGSESKYGPPCPPCPASTTCIPSSGHSRHRYALIPIPLAVITTCIVLYMNVL

SEQ ID NO: 10 - DNA, 1002 bp, synthetic construct
  source 1..1002: mol_type = other DNA
atggaaaccgacacactgctgctgtgggtgctgcttctttgggtgcccggaagcacaggcgactacccttacgatgtgcctgactatgctggcggcggaggatctggcggaggtggaagtgatatccagatgacacagagccccagcagcctgcctgcttctctgggagacagagtgaccatcaactgccaggccagccaggacatcagcaactacctgaactggtatcagcagaagcccggcaaggcccctaagctgctgatctactacaccaacaagctggccgacggcgtgcccagcagattttctggttctggcagcggcagagacagcagcttcacaatcagctccctggaaagcgaggacatcggcagctactactgccagcagtactacaactacccctggacattcggccctggcaccaagctggaaatcaagagaggcggaggcggtagcggtggcggaggaagcggaggcggcggatctgaagttcagctggttgaatcaggtggcggcctggtgcagcctggcaagtctctgaagctgtcttgcgaggccagcggcttcaccttttctggctacggaatgcactgggtccgacaggcacctggcagaggactggaatctgtggcctacatcaccagcagcagcatcaacattaagtacgccgacgccgtgaagggcagattcaccgtgtccagagacaacgccaagaacctgctgttcctgcagatgaacatcctgaagtccgaggacaccgccatgtactactgtgccagattcgactgggacaagaactactggggccagggcaccatggtcacagtttctagtggtggtggcggcagcgagtctaagtacggacctccttgtcctccatgtcctgccagcaccacatgcatcccttctagcggacacagcagacacagatacgctctgatccccattcctctggccgtgatcaccacctgtatcgtgctgtacatgaacgtgctgtga

SEQ ID NO: 11 - protein, 250 aa, synthetic construct
MVAGSDAGRALGVLSVVCLLHCFGFISCFSQQIYGVVYGNVTFHVPSNVPLKEVLWKKQKDKVAELENSEFRAFSSFKNRVYLDTVSGSLTIYNLTSSDEDEYEMESPNITDTMKFFLYVLESLPSPTLTCALTNGSIEVQCMIPEHYNSHRGLIMYSWDCPMEQCKRNSTSIYFKMENDLPQKIQCTLSNPLFNTTSSIILTTCIPSSGHSRHRYALIPIPLAVITTCIVLYMNGILKCDRKPDRTNSN

SEQ ID NO: 12 - DNA, 753 bp, synthetic construct
  source 1..753: mol_type = other DNA
atggttgctgggagcgacgcggggcgggccctgggggtcctcagcgtggtctgcctgctgcactgctttggtttcatcagctgtttttcccaacaaatatatggtgttgtgtatgggaatgtaactttccatgtaccaagcaatgtgcctttaaaagaggtcctatggaaaaaacaaaaggataaagttgcagaactggaaaattctgaattcagagctttctcatcttttaaaaatagggtttatttagacactgtgtcaggtagcctcactatctacaacttaacatcatcagatgaagatgagtatgaaatggaatcgccaaatattactgataccatgaagttctttctttatgtgcttgagtctcttccatctcccacactaacttgtgcattgactaatggaagcattgaagtccaatgcatgataccagagcattacaacagccatcgaggacttataatgtactcatgggattgtcctatggagcaatgtaaacgtaactcaaccagtatatattttaagatggaaaatgatcttccacaaaaaatacagtgtactcttagcaatccattatttaatacaacatcatcaatcattttgacaacctgtatcccaagcagcggtcattcaagacacagatatgcacttatacccataccattagcagtaattacaacatgtattgtgctgtatatgaatggtattctgaaatgtgacagaaaaccagacagaaccaactccaattga

SEQ ID NO: 13 - protein, 33 aa, synthetic construct
TTCIPSSGHSRHRYALIPIPLAVITTCIVLYMN

SEQ ID NO: 14 - DNA, 105 bp, synthetic construct
  source 1..105: mol_type = other DNA
acaacctgtatcccaagcagcggtcattcaagacacagatatgcacttatacccataccattagcagtaattacaacatgtattgtgctgtatatgaatggtatt

SEQ ID NO: 15 - protein, 220 aa, synthetic construct
MLRLLLALNLFPSIQVTGNKILVKQSPMLVAYDNAVNLSCKYSYNLFSREFRASLHKGLDSAVEVCVVYGNYSQQLQVYSKTGFNCDGKLGNESVTFYLQNLYVNQTDIYFCKIEVMYPPPYLDNEKSNGTIIHVKGKHLCPSPLFPGPSKPFWVLVVVGGVLACYSLLVTVAFIIFWVRSKRSRLLHSDYMNMTPRRPGPTRKHYQPYAPPRDFAAYRS

SEQ ID NO: 16 - DNA, 663 bp, synthetic construct
  source 1..663: mol_type = other DNA
atgctcaggctgctcttggctctcaacttattcccttcaattcaagtaacaggaaacaagattttggtgaagcagtcgcccatgcttgtagcgtacgacaatgcggtcaaccttagctgcaagtattcctacaatctcttctcaagggagttccgggcatcccttcacaaaggactggatagtgctgtggaagtctgtgttgtatatgggaattactcccagcagcttcaggtttactcaaaaacggggttcaactgtgatgggaaattgggcaatgaatcagtgacattctacctccagaatttgtatgttaaccaaacagatatttacttctgcaaaattgaagttatgtatcctcctccttacctagacaatgagaagagcaatggaaccattatccatgtgaaagggaaacacctttgtccaagtcccctatttcccggaccttctaagcccttttgggtgctggtggtggttggtggagtcctggcttgctatagcttgctagtaacagtggcctttattattttctgggtgaggagtaagaggagcaggctcctgcacagtgactacatgaacatgactccccgccgccccgggcccacccgcaagcattaccagccctatgccccaccacgcgacttcgcagcctatcgctcctga

SEQ ID NO: 17 - protein, 27 aa, synthetic construct
FWVLVVVGGVLACYSLLVTVAFIIFWV

SEQ ID NO: 18 - DNA, 81 bp, synthetic construct
  source 1..81: mol_type = other DNA
ttttgggtgctggtggtggttggtggagtcctggcttgctatagcttgctagtaacagtggcctttattattttctgggtg

SEQ ID NO: 19 - protein, 12 aa, synthetic construct
ESKYGPPCPPCP

SEQ ID NO: 20 - DNA, 36 bp, synthetic construct
  source 1..36: mol_type = other DNA
gagtctaagtacggacctccttgtcctccatgtcct